European Patent Specification EP 3 673 910 B1, published November 22, 2023. Title: Sugar chain-related gene and use thereof. Applicant: STELIC INSTITUTE OF REGENERATIVE MEDICINE STELIC INSTITUTE & CO. Application not yet assigned. The sequence listing filed with the application follows.

SEQUENCE LISTING (98 sequences)

SEQ ID NO: 1 - DNA, 9120 bp, Mus musculus
tgtatatctgagtatctgtgtatgtgcatatatgtgtgtctatgtgtatgtgtgggtttgtgcatgtgtgtctgtgtgtacatgtctgtgtgtctctgtgtgtgtctgtgtatgtgtgtttacatgtgtgtgtgtgtttctgtgtggacgcatgtgtatgtgtctccgtgtgcctgcatgtgtgtttgtgtatgtgtgtaggcatgagtacatcatggtgtacatgtagaaattgagagagactcttgggtgtggttctcatctcccaccatatctgaagtaaatgtcttattcacaccactgtgcacatcagaaagctagccttgacctccaaggaactctgtctctgtctcctgtcttattgtaggtacctggggtttataagcctatgctgctgcatatggcttcacttgggttctggggatttgaacttaggtcctcacagttttagggcaagcattttattcactgaacaatctcccatgatccctagagtttattgtaggcaacttaacctttagtcgtcattgagatttagcattgatttcagttccagttgtattctgatgttgagcgctacagcagaggtacccagggactgctgattttctgtggccatgaatcctctagtgattaataaatttcatcataatgttctgtttatttctaaatgtccagacaactctaatttcaaattaatctcatcctaaacagcacaggataaaagttacagattgtcctatcttcattcatgtgatgcctcaaatcagatgtttaatcctttagtcagttatttgtgaaacggaacctaattacacacactcgcatgcgcgtgcgcgcacacacacacacacacacacacacacacacacacacacacacttgtagatttgcccacacagctgcttaagcaatttggagcaaatgtagaaatattatgaaatttcacataaaaatgggttttcctctgtcttcttgagaaatgtgtgagtttcaatatgacagtaatcttctggtgttggactataaccacttgaacccctgaggtactaagtgtgtacctactacgtgcctggattccatcatttccctacttatataagcttctccatcctgtagatcagcactgtgtaatggagtaacacaagtcattgaatcatgcaatcatttaatcaatttaattggcacttctgataagagaagtgggcacatatttagttgtgtttgcagcctgtgctatgtcatttttctctatatatactttaagatttttttcttttttccatttacggggggggggttattccatttaatttacatgcttaatgacatataatttgcatatcaggtgttcctttctttagagttaacttcttttaggaccattgtttataatggatgtatatcatccctaaattaaatcagccattgtctacttaacacaccagtttctctgatgtccctctggctcttcctcctctgaggttctagttataggaaagtctggcattttgatgtttttccatggcttcgtgggctctgatcatccacttacagtgtactttcatctcttgtctacaaactgcatatcatctattgatctgcgttcaaggctactacattttcatgcaattccactttgctgttaaaccttttctatgatccgtttttatacttataaacaatccaagtgttgtactctttgggtataaatgttctgtatttcacaggtcttaacttcttttcagactatacaaagaaagattttctattttttttatttgttgtatgcattttatgcatttagcactgggatttccataacaggcagttaagatcattgaatacatactttgtgtggtaaatataatacggcttatttgattctcccccttaaaatgctcccatcttctcagtcatgtcaggttgctatggagtccaccctgagcaccatgagtgtgatgctgtacagacactcctgatatgccttctgttatttgaactccacctgcaagttttcattcaagcatagctcctaatcccattcagtgtgcacttttcttaattgatttgctggtagagagctatatgtaagcatggcttagcatcaaattgaactttctcctctccctagcttctttccagtatattcttcctcaccttcatcagattttgaggtcttgagatctaaaccttcatgttacaatttgcagagataccaggatctctatcagacttgatgtgtctccatgtaattctagtatcagcctttcataagataattgcaaaatatagaaccccccctctctccttttgactattacagctttgtttctctcccaagttaatacagatgtatgcaaatcaactaagaaaagcaaacactgaatgggataaggagctatactcaaaagaaagcttgcagttggagttcaaataacacaagtggaaccaagagtatctgcacagcatcagactcactgtgctcaggatggaatccatagcaacctcccataactgagaggatgtgagccccttttaaagggaaaatcaaataagcagtattatattaaccacatgatgtgtatattcaatgtagattgggctgcaccgaagttatgattttagtaatgagtatttctccttgggttttcttctggaccaccctggttttccttttaaaaatagtaaaatagcagcaatgactgcttctcttaaaatctgaacaacacagagcacttcagcatcctttcaacctatctaaatccattgtagacctgcactgacttgctgtgagctattgtgtcacaactattattgtagctaaacaccttgaattttcaaagctgctctggactgtgtcttcttttagaattaaacttgctaaagatattggactctgagatgcttattcaccactttctataaaagagtaaggatgacaatgctttgagtagaagaagattgcatacgagggtaccagcatgtcattatgtccccagcagtcagtaaagtaaggatccagtgatggtagagttattatgtccattatggaactaatgtaaatgtttatcaatgactagaatggctgtaatcaccaatccttagacaagtgtgagtaacatcatgctcttttcttataataatagatagtcacacacaccatggtcttaaacattacattttgatttttctctttgtgtctgtcttttcgtacctctactccacttacctgagccttcagctagggctcctccaagacggcagtcacagtactagtgaggataattctcatatggagacctgaagcagaataaccttcttccaaggaaaccaaaatcctagtcaacatcttctccactctttggttatttatttttatttctatttctattttgccatttaagaatttttaaactcttttctgttttcttatatatattcttttttttacaacttttgatattctttatcaaatgatttatcccattgcctttcctcctgcagctatctgtgagttttagcatggatatttagaatacaattggaaattatgaaggtcgaataaaagttctctaagagccaggacctcactagcctagttagttgcttagtttctaatataaggcatggtttatctcctactgtatggcccttaaatccactagacatctgttggcttccaacagcatacaattgctgctattgtatgtttaggtatatatttttatgaaacactatattctgattggtgttcattcttcctatgaaggggaagattttattgcctgctcaaattcaagtcagtcctttttgagtagacaaaggttgtccaatcttgctaaacccttttcttttttgcttggggaatttctttagggaaaattctcaaccatgaaccaagcctagagattgataatagctgaaggcagagtagccagtcttagtaagggatgagagaaagactgaccaaagactgaataggaaatggttgatagcattcattgggactagacaataaagttagctaccccaacatgggcaaatggagaaaatggggagagtcatatggatatgtagggaggagaagaaaggaaggggtgagtttgaagtatggaagagcctttaaagcatttgtaagatttgtaagaaaaagcttttgagagacagagtattacctgccttcaaatcccttcaattactgtccctacaagacatacctgtgctcagctgctcttggaccacaagggggcctaagagcatgtttgtgtccctgtctttatacaggcttctcatctgtatttctcaaacgtaaatacaaatgggggagataacaaatgatatttctaagtggtacacaggtatgagaactgcacacaatctatttatatgtataatggccagagctctcagcagggaacagaggaagcctaggtaactcctgctccagagcatgtctgtatggagacctcagttcagcaactatgaaatctgtgttcaaagggtcatcactgggaacagtttctggaatagcagacatattcattctctctctctctctctctctctctctctctctctctctctctctctctctctctctctgtctgtctctgtctctctctgtctgtctgtctgtctctcccttctgtcaggggtatgcatacatgggctgggaattctatcttccctgcctgctgtctttggtgtctccctaatgtggtgccatgtttacttaacctgtctgaaatggaggataacctctggtctgataactgtcaagttactgaaatgtcagggaattgtgaatgaacccctctgaatgctgggcagatgttttgagcacgtgggtatccatagatttttttttcagcaggatttccttctttaatatattgtgggaacgaaacattgaagtttccaacactaagaaaagcaatgctctgggtttgcaaagaagtctccaaagctgtgggagaggcaatggctttgcctcacaaaggtgatcctgatttggattgggtgttcctcagtctccctcatcctttgtttgtggaccaaacctctgatcaaataatcagtatacagacaagtactgactgactcctgtcactgtttcccatgtaaattctcaaccatgtgtgtcagaattgtttgagtcatcaaagttccgtgatgctcaggatggtgaataccagaaactgaagtctgaaatccaatttggcctttctcgggcactgtaaactgagtgcaaatgtgcccagttccctcgtggcccatttatagcacaataacacagtgcttgcttacaaaatctagtcccgattaaagtatttatttaaagttgctttagacaaatatatttctaaatggaaggatgaaacagaaagaatattccaactgtacagtctatattttgtttctaaaaatttttattagaattctgacttttagaaaacaaatagatattcaaaaactacttctttaattaaataataacatcattatagacattctccagccatttagaagtagcatgattacaaagcattcatgttccctttgttttttgaaacagaagtatttatatgacaaataaaaagcaaaaatctcatatatgtgatagctatagatgcattgataggaattaaatttaatcaaaaagaacttttaatggcaataatgtggctactaacttcattgtttgtaataatgctgcaaatgtttaatgaaaactgttactaacaatacaggagaagattacagatatgattaggtcgtgttgatagaaatggaaagagaaaggtcactcactacctcagccacagaacttgaggaatgtgtgagggtttttgaggaaaaaagagaacaatgtaacatcacagcaacatcttaatctgaaagtagacgacaaaggtttcagagtaggggatcagaaatttaagtatgcagagaagcaaggcatatacggcttagacaatgtatgaagaacagcagcagacagcaagtgaaagaaatcacagtccacatggaaatcacacagaccacagtgtgcacacagagacagaaatcagcaagggacacacggcttccagttatgaaagttagacagcaaaatttaagttgtcccacctaaaacatgatgtatcgtctctcaaatggggaaggggaaggagcagcaaacatctggatatgtctaaaacctcacagagaacatctgggatctttgcatttctccctctgactttctcaatatgttagctacttctagatagtttcaataatggtctctaattgactatggagagacaggtctcatgtatgtgaacatccttaaccaggagatggaatgtgtttccttgtcactcattttctaaggaagtgaattccttctgcattgcccaggattggatgttacgtgaaactaaaaatcattgattaaaaagaaatgtcattaccacagttgggttgaatcaatcaagacttatcctagttacaggcatcacctccccttaagcacaaatactgagaacagctaagctcactttgaaatctgggatgaggaggctttaggtcaagcatctgacaatgtgtgtgtgtatgtgtgtgtgtgtgtgtgtgtgtagtatgattatatgtatatatgtagatgtgtgtatatatttatatgtatatatgtatatgtgagtatgtatatatgtatatgtgtgtatgtgtatgagtgtgtgtatgtatgactatgagtgtgtatgtattgtgcaagtgtgtgtatatatgtgtgtatatgtttatgtatatgtgtattgtatgggtgtgaatgtattatatatgtgtgtaggtacatatgtgtatatgtttatgcgtgtatatgtgtatgcattatatgtatgtgtgtatgtgtgtatgttttcatgtgtatgtagcatatgtatatgcatgtgtgtgtctgtgtgtgtaagcatgtatttactaagaaaaaatcagtttctctagctaatgagtcattgaagtgaagaaaccttacgctatcacattactatgtttccagcataaattgcaatatcagtaagacattccccatcataacttaatggacacttagattaggtcatgcagcagtaaattatgaaagcgtctatgctgagctgaggtgggaaatcgtctttcctgcctccttcctcctgttctttctcctaaaggccctcatcctctttctccccttcctttcttttaaaatattctatcattgatccaagctaactaacccttcccttgctcacatgtgacctgcccagaggaatctatttatagtcaacaataacaggccaaggacatgcgaacaaatgactttacttagccccacttggtgaatctattgggtgaataggtaaggggttatttataggagcttgactgactggcacagctgtatctctgaaaagtcccccaaagcatcatgggtgggaactaaggaaagccggaaatgctggagctggaatcccaacctgcagtggctacatgatgaatgtgtctcctttcctactaaatatttaagactctgggcaggctggttagtcttgtaaaagtcttgtgggtttctggagtcctgggaggctcactgtccctgcagaagcttgttattattgtatatgaaagaaagtgctcaacactgagtcacaaaagaagcccccgagaatcggtggcagaggtggaaatagaagaatccgatgcagttcccgaggcaagagttgatcctctccatggtgacaagaaaacaagagccacagaagcctgaaggctaagactatgacctgtgaggttctcctctcctaggacttgaatgcacttaactctgagggctagcagggcagagattcaggagcgttctcagaggttgtcccttctccttgtatgattctaggagaagctcagtgcataggcagaagttgcaaactctaacacattaacccacatcctgaattgttttatatcaattgttttataactacatgttttaacttttgttttggtttttgaattttgtttgtttgtttgttttctatttttcatatgtgtgcatgtgagccagaagacaggctaagggactctgttctctctttccagcatgtgggtttcagggatcaaagttaggtcccaaggcttcactgggcaacgggacccttagcctctgagtcatcttcttaatctttttctttgaaactttttcattacattgtgtcagtgcacacacacacacacacacacatgcatatacatccacatgcatatacatccacatgccatatgtcatggcacatgtgtggaaagaaatgggtgccttgaggaaatcagttttcttcttccatcacgtggatcttatgacttcaggtaacccatctctgctccccaagcatggctacaagcatttacctgccaagtcatctccctggctcccacattaatttataataatacaccctttcagcctagagagatgactcagtggttaagaactctggctgtgcttcagaaggttctgagttcaattcccagcagctataaggtggctcacaactatctctaatgttgttttctgtcctcttctggcatgcacttgtatgtgcagatagagtacttatatgcataaataaatataaatacattaataatcttttaaaaagaaggaaagattaaaagaacaatacaccctttcttttaagtaagaaaacatgcttagtatatagaataaatgctggtgttgaaaggtgaaattcagaagaaattataggttggaaatatttgaactcttttgtgtcaaaccaaatggtaaagatgatgtgataataaggtaaggttttcttcctacacatatacttgtttaataaccagtataagactatgagtgaacataactaaaaatacatgaaaaaaaactattttaaaaaaacatcactttcagatgactctggtgaaactcactgataaccagcaatctctttgatagaccagagtgtccagtctgaagttaattcttttgctttattctcaaacaatgttgcagaagtatgaaccatagtatcaagatacactgtccacatatgcacctggcctgacttgtgt

SEQ ID NO: 2 - DNA, 2105 bp, Mus musculus
  CDS (418)..(1671)
gagccttcccggcgcgtgagccggatccggtggcaccgcggggaagagacaggaccgggcggtggcggcagagacagggggacgcacccggtgcagaagatccaataggagcacgccgccgcaacctctcccgcgcgctccggtcgccgactctacgccgatcgcccactccccgcaccttggactacaccgggaaaaagacgcagcctggcccgaactggggcggagatccttcttgcttcccaagagctcgggagggaagattctcccgccgccgagaaccccgccggactggaggaacccgtggcctggagagcgctggctgtgccagaccccagcctgatggatgtctggtgtggataatgagggaagaacgtgccttttacacccaagaggtgaccccggagcgtgccccggatgaccccacaactcggaacgatgcggctagcctgcatgttctcgtccatcctgctgtttggagctgcgggcctgctcctcttcatcagcctccaggaccctatagagctcagcccccagcaagttccaggtataaagttcagcatcaggccccagcaaccccagcatgatagccacttgaggatatccacagaaaagggcacacgagattcacccagcgggtcgccaagaggcctccagctgcaagcgcctgaccaacctcgacctcacccgaaggcagcgggatctcctttgcgcctccggcagcgcaggcggagactgctcatcaaaaagatgccagccgcagggactaaccaaggcaacaactcgtccgaaacctttatccagccgagaccccgcaccatggacagtcgttgggtcagcctgcaccagacccaacaggagcgcaagcgtgtgatgcgagaagcctgcgctaaatacagggccagcagcagccgcagagctgtcactccccgccacgtctcccgcatcttcgtggaggaccgccaccgtgtactgtactgtgaagtacccaaggcaggctgctccaactggaagagggtgctcatggtgctggcagggttagcctcatccacggcagatatccaacacaacaccgtccactatggcagcgcccttaagcgcctggatacttttgaccggcagggcatagtgcaccgcctcagtacctacaccaagatgctctttgtccgggaaccctttgagcggctggtctctgctttccgagacaagtttgagcatcctaacagctactatcatcctgtctttggcaaggctatcctggcccggtaccgcgccaacgcctcgcgggaggcactgcggactggctccggtgtgcagttccccgagttcgtccagtacctgttggatgtccaccggcccgtgggcatggacatccactgggaccatgttagccggctgtgcagcccctgcctcatcgactatgactttgtgggcaagttcgagagcatggaagacgatgccaacttcttcctgcgtctcatccatgcgcccgggaacctgactttcccgaggttcaaggacaggcactccgaggaggcgcggaccacatcgagaatcacccatcagtacttcgctcagctctcctcgctgcagcgacagcgaacctacgacttctactacatggattacctgatgttcaactactccaaacctttctcggacctgtactgagggcggggcctgctggtcaggggcggggtctgccggtcatgcccactcacctgcgcataggcggcctccggggactgagctctgaggatgtgaggccttgtggctgtggccctagggtgggccacagaggcccagacaatggaccttgacccttgtcccacacccatttcctcattgggttggctgagtttgagacggagcacgactcggatggatgctttaagaactcagctgagctatgctgagctatgctgtccagggaagcctgagacccagaagagggccccagcgtcgagggatgtcctacatccccttatcctttgccttgtaccaaaccacgtggtttgctgcttttctatgacccagggtcatctgaataaagcacatggttttcagagcaaaaaaaaaaaaaaaaaaaaaaaaaaaaaaaaaaa

SEQ ID NO: 3 - protein, 417 aa, Mus musculus
MTPQLGTMRLACMFSSILLFGAAGLLLFISLQDPIELSPQQVPGIKFSIRPQQPQHDSHLRISTEKGTRDSPSGSPRGLQLQAPDQPRPHPKAAGSPLRLRQRRRRLLIKKMPAAGTNQGNNSSETFIQPRPRTMDSRWVSLHQTQQERKRVMREACAKYRASSSRRAVTPRHVSRIFVEDRHRVLYCEVPKAGCSNWKRVLMVLAGLASSTADIQHNTVHYGSALKRLDTFDRQGIVHRLSTYTKMLFVREPFERLVSAFRDKFEHPNSYYHPVFGKAILARYRANASREALRTGSGVQFPEFVQYLLDVHRPVGMDIHWDHVSRLCSPCLIDYDFVGKFESMEDDANFFLRLIHAPGNLTFPRFKDRHSEEARTTSRITHQYFAQLSSLQRQRTYDFYYMDYLMFNYSKPFSDLY

SEQ ID NO: 4 - DNA, 1369 bp, Mus musculus
  CDS (40)..(1281)
attcagacatgaagagagacacagtggtctgaagtggtcatgaaagccaaacaagtcttcttttctgtcctgctgtttgggacagcagggcttctgctcttcatgtacttgcaagcatggattgaagaacatcatacagggaaaatagagaagaaaagggatcagaaaggagtatcggtgactacgggaaaaatccagaaacagatcacgaatcagaactctgaggttcacatgcctgaagatctgaagaagaaagggggagatctgctcaacctagggagtccaacaagggttttaaggaagatcagccattcacaaagggagaacggagcttacagatcaactgaagcacatcaaggagctaaaattgaagtttttcagaaacccatccagatggactggccactggtcactcagcccttaaacaaaagtttggtccaaggcaacaaatggaagaaagcagatgcaacccaagagaagcgtcggtcattccttcatgagttttgcaagaaatatggtagagtaaatgatcccaagttcaacctttttcatatagtatctaggatatatgtagaagacaaacacaaaatcctgtactgtgaagtaccaaaagctggctgctctaattggaaaagaattctgatggtcctaaatggattggcttcctctgcatacaatatctcccatgatactgtgcactatgggaagcatctgaaaacactggatagttttgacttaaaaggagtacacatgcgtttgaatacatataccaaagctgtgtttgttagagatcccatggaaagattagtctccgcatttagggataaatttgagcatcccaatagttactaccatccggtgtttggaaaggcaattatcaagaaatatcgaccaaatgcctctgcagaagcattaaataatggatctggagtcaaattcaaagaattcgcctactatttgctggatgctcaccgtccagtaggaatggatattcactgggaaagagtcagcaaactgtgttatccgtgtttgatcaactatgactttgtagggaagtttgagaccttaggagaggatgccaattactttctacagttgattggtgctccaaaagagttgacatttccaaactttaaggataggcactcctctgatgaaagaaccaatgcccacgtggtaaggcagtatttaaaggacctgagcacagccgaaagacagctcatctatgacttctatcacttggactatttgatgtttaattacacaactccacatttgtaatttgcattcatttttctaaagccctacatagatttaatgatgatggcctcaaataagctactgtaattgtcctacaattctctgtatg

SEQ ID NO: 5 - protein, 413 aa, Mus musculus
MKAKQVFFSVLLFGTAGLLLFMYLQAWIEEHHTGKIEKKRDQKGVSVTTGKIQKQITNQNSEVHMPEDLKKKGGDLLNLGSPTRVLRKISHSQRENGAYRSTEAHQGAKIEVFQKPIQMDWPLVTQPLNKSLVQGNKWKKADATQEKRRSFLHEFCKKYGRVNDPKFNLFHIVSRIYVEDKHKILYCEVPKAGCSNWKRILMVLNGLASSAYNISHDTVHYGKHLKTLDSFDLKGVHMRLNTYTKAVFVRDPMERLVSAFRDKFEHPNSYYHPVFGKAIIKKYRPNASAEALNNGSGVKFKEFAYYLLDAHRPVGMDIHWERVSKLCYPCLINYDFVGKFETLGEDANYFLQLIGAPKELTFPNFKDRHSSDERTNAHVVRQYLKDLSTAERQLIYDFYHLDYLMFNYTTPHL

SEQ ID NO: 6 - DNA, 5532 bp, Mus musculus
  CDS (369)..(1427)
ccagtgcacggcggcggcggcaccttccttctcgcatcccggtcgcccggcccgtgaggaggcagcggcggccgcaggcgccagcagaggaggcggcggagcatcgagcagaggcgaggcggaccggcaggagcgcgcggccggagccacgcatcctcacacttgcacaccaactcctgcgcctttcaccctctagaccagagtcggggcctcggagagcctcggtgaagctagcgggagccagctccggagcccagccagctctgttctgagcctccccggtgctggtacccccgcggcggggtccccgcttctgcgctcgggacgcgcctcccggacagccgggtccccgcggccaggacaaagccatgaagccggcgctgctggaagtgatgaggatgaacagaatttgccggatggtgctggccacttgcttcggatcctttatcttggtcatcttctatttccaaagtatgttgcacccagtcatgcggaggaaccccttcggtgtggacatctgctgccggaagggatcgagaagtcccctgcaggagctctacaatcccatccagctggagctatccaacactgccatcctgcaccagatgagacgggaccaggtgacagacacctgccgggccaacagtgccatgagccgcaagcgcagggtgctgacccccaacgacctgaagcacctggtggtggatgaggaccacgaactcatctactgctatgtgcccaaggtagcgtgcaccaactggaagaggctcatgatggtcctgagtggccggggcaagtacagcgatcccatggagatcccagccaacgaagcccacgtgtcggccaacctgaagacccttaaccagtacagcatcccagagatcaaccaccgcttgaaaagctacatgaagttcctgttcgtgcgggaacccttcgagaggctggtgtctgcctaccgcaacaagttcacgcagaagtacaacacctccttccacaagcgctacggcaccaagatcatccgacgccagcggaagaacgccacgcaggaggccctgcgcaagggggacgatgtcaagttcgaggagttcgtggcctacctcatcgacccccacacccagcgggaggagcccttcaacgagcactggcagacggtctactctctctgccacccgtgccacatccactacgacctcgtgggcaagtatgagacactggaggaggactccaattacgtactgcagctggccggagtgagcggctacctgaagttccccacctatgcaaagtccacccgaactaccgacgagatgaccacggagttcttccagaacatcagcgccgagcaccagacacagctgtacgaagtctacaaactggactttttaatgttcaactactcagtgccaaactacctgaagttggattagagggctgcggaggggagggggaggggtggttgggggagagggagagaatcctgctttttaatttaagatttttatttgtcaaaagaattctatggagactgggttattttgtaagttaatatgtcttcgggggagatgctgcgagcggcatggttaagaattatttaaaaattctccacggggaaggacagctgtctttgcaggggagcggggtggaatatccctgtttttagaagtggatactgcaacactgtctccaaggtgtccttgtgttctggtgaagtccacaaactgcattccataaagtctaatgaatcttatttatagttatttaaacgtggtctgtggcagcagcctgctcctgtctgtgcagaggagagtacagtctgtgcttcgctggctatggctcattgggggaggggagggggttatctcccccactgaccgtgtgtagaatcccatggtgacagctgcgggatgtgtgcctgtggccattcaagaaaccctgctagaaagaagtcaattgtccttgcactaagaaacagggatgagactggttcaaaccgattgctagcaaccccaaagtcccttgtagtaaagaaatgcaaatttttttaacccaagaagagagcagatgatagcgatttctctttaccgaaattagcaggctataagaataggctttctgtggaaatctttaagtggcactttccagtgctagcgaaggcagaataatggttgttttctagtcaataagtattgagcatctactattctccaggcttgactgcagatagcacattgagtgaaaccaggagccttggccttcagcaagctttatgtgaacacagggcatccagctcaacagtgaaccaacacccccatccctttggtcctcacacagactttagactattctcaagtggtccagagggtccaggaccctagcaaatttgcgtatttctacagttcaaatttgaaagccacacatttggatcaggccacttaactagctaagtagttcattgcccaacacaagaaatgacagaaacccttttgatcatgtatatctagtgcagtgtcttcatagtagaagcctataagccacaatattctccaagcgcaaggatggaggactgctgtgattgattagtgatgtctgccttgactaaggaaagggaggaacatttctcaagggcctcctactgtgatctccagtccacatcttgtcctgcctgccacttaaaacagtgcactgcatacatttggagactggcggagttcaagtgtgaaggtcaaaggtggagtgttggtacccacaggcacatgcccaccctccatgtcctgcattggcagagcatccaggacctccctctcctccagaaggttggaaatttgctctttcctgttccttgctgatcaatgcccaaacctattcctcatttctagttgtttctgatactttgcggttgacatttgagccacattcccatgacagccagtgtccgggtacgtagcagatgctgtacatagttctgatgataagggagctggtaggctgtaaattttgctttttgtgtttttgtggggttttgtttgttttgatgcagtatagagtgaagggggtaagaatattctgaaaaacataaaattgagtaatttattcacagaaactattaaaatggtattgttaggctcacaaggaggctgggggcagcggtaactgctacactgtctcgcagaggaaattattttatttaatgtgagagaaatgtgagccagagtggctgcctgaggctatttataaaacgcaggtaccttccccaatttctctcccctcgcctttaataaatagatttatgtcatgtgtgtgaccaagaacagtgacagatcttggctgtccctggaatagagaggcagtcatggtgctcaggccctgggcgtggtgtagctgatgcatgtcccaccgagcccaggctctccaaggcatcagtttgtggtcacatatccttagaaaacaaaattaagtcaggttcctgtctgcaggagttttcagagccttgaatacatagtctgccttgtgaaactgggagaatgtagcatttctgggctgcatgacctaggtatcctgtatggcagaccatgtcttagctggtttttcacacagtagccttcagtgagggtgatctagcctgtctgaggtctgcaaagattgacagctgcttcctagatccttccacaaatcagcagaaacagtgtccatctgggaactttatgagagtgttgctttacctagttggggtgtcttcatctggatactgccccagagagtgatcccgtccctccaagcacagcggagggaagcctagggtgttatggagtggggcaggtggcttaaggacaccttaaaggccacttggtggggataatggcctcgtggggatactcctcacttccacccacagtttggaactgttcactgtgtgcttcaggagttttaaatggagattcgtgttgatttccatggtccgcatctgtttgtcttccgtctgtggtccagtgctgtgtgcagatggtacttactccctttctctctcttacagggagaaagactgtccttctggggagagtgtatcaatacgcttccagaatgagggagtctttctcctgtcttgtgttcacacttcctagtgacaattttcaaaatatgtatcggcttgactgtttattgtagagtgtagaaaggtttctgtgttcctggctaaagacatccattggtgaaatgtgcttggaaatccaagtgttttctactgaggaaaaaaaaatgttggaaaagctttctcctgcatgcctcttgtgcttagctagaaaggggagctgccagcgtcccagctctgagccactgttcaaaggtgcagctgtgttttaggactaggtacaggcagagtgataaggacatgcctgcttagtgtactcatttatcgagaaagtttagactatgagccacaggggtccctgcctgcagtccctatagcctccccctgccccagtgcctttctcagctggtctgggaatcagggcagcccattgaggggggctcagacaaccctttcttcctggttctgggagtaaggctttctctgcagccacaaggagaacatgggaaccagaaacttctctttggtcagcccttctgagcacacaggtttagcccatgctccaagaatgctcctgagcattgtataagcccctaggactcttagctcatgtgataatgattgcattactatcctgctttaactgacaaaaccacagagaattttgcttgctttcctactctcttcctctgcccaggcctcctccatacgtatacatacacacatgggcatgtatacacacacatgcacaatagacatgcacacacacatgcacacatgggtatacatatacacacatgcacaatagacatgcatatatacatatacatgcacacattgataggcatacacacatgcacagtagacatgcacacatgggtatacatagacacacatgcacagacatgcatacacacacatgcacacataaatgtgcacacacacatacacaaattgcccaagcctgtgcactcctggtacccatgtcccatcctggcccacctctttgtcagcaggactgactccatcactccctcaggttttgcccaccagcaccccccagctttcccccagcagagctaaacagcccctctgaatagacaacaggaccttctagaaacagctgaacccttggacagcagcaggcagattttgatctgctctcatcaggtacaaaaggtggtatccgtattctcttctgagcatgctcagtaagcatatggacatagaatttaacatctctgtggagtgtgtgttttttacatatttgtatgcagtcgaggagggcctgttgtagaattctctccctgtatcttactatactgttaaagaagctgaattctatgttgccaacagatgcgtgaaatgttcctccaggaaaagccattcaagcctgattatttttctaagtaacttcaattaaattgaagaagaaaaaaaaaaaaaaa

SEQ ID NO: 7 - protein, 352 aa, Mus musculus
MKPALLEVMRMNRICRMVLATCFGSFILVIFYFQSMLHPVMRRNPFGVDICCRKGSRSPLQELYNPIQLELSNTAILHQMRRDQVTDTCRANSAMSRKRRVLTPNDLKHLVVDEDHELIYCYVPKVACTNWKRLMMVLSGRGKYSDPMEIPANEAHVSANLKTLNQYSIPEINHRLKSYMKFLFVREPFERLVSAYRNKFTQKYNTSFHKRYGTKIIRRQRKNATQEALRKGDDVKFEEFVAYLIDPHTQREEPFNEHWQTVYSLCHPCHIHYDLVGKYETLEEDSNYVLQLAGVSGYLKFPTYAKSTRTTDEMTTEFFQNISAEHQTQLYEVYKLDFLMFNYSVPNYLKLD

SEQ ID NO: 8 - DNA, 1785 bp, Mus musculus
  CDS (149)..(1408)
ggcgatttcggctgcagaatcagcatcaccagcaacagcagcagcggcggtgactgtggcgggcgctaggtccgtctcctagggaccatgtcccagctgtgcacaaggctgaagtgaagggccaggagtgggcccagcccagggcagcatgaccaagccgcggctcttccggctgtggctggtactagggtcggctctcatgatccttttgatcattgtatattgggacaacgtgggaaccgcccacttctatctgcacacgtctctctccaggccacacatcctagaaccccttcccacccagggattggtggaggagaacgtgttcacatctgacgtggatgagtttttggatactctccttagttctgacgcgaagcacaacgacctttccaggagaaaaactgagcagcccccggcgcccgcccccagcaagccagtcttgagccacatggaggagaacgtgagaggctacgactggtccactcatgatgcccatcagaaccctgaccgggacaggcagcaggccgagaggaggagcctgctgagagacttctgtgccaacgccagcctggcattccccaccaaggaccgctcttttgacgacatccccaactacgaactgaaccacctgatcgtggacgaccgccacggggtcatctactgctacgtgcccaaggtggcctgcaccaactggaagcgagtgatgatcgtgctgagcgagagcctgctggaccggggcagcccctaccgagaccccctggacatcccccgggaacacgtgcacaacaccagcacgcacctcaccttcaacaagttctggcgccgctacggaaagttctcccgtcacctcatgaaggtgaagctgaagaagtacaccaagttcctgttcgtgcgcgacccctttgtgcgcctcatctcagccttccgcagcaagttcgagctggagaacgaagagttttaccgcaagttcgcggtgcccatgctccgactgtacgccaaccacaccagcctgcccgcctcggtgagtgaggctttcagcgccgggctcaaggtctccttcgccaacttcatccagtacctcctagacccacacacggagaagctggcgcctttcaacgagcactggcgacaggtgtaccgcctctgccacccgtgccagatagactatgacttcgtggggaagctggagacgctcgatgaggacgctgcccagctcctgaggttcctcaaggtagactcccagctccacttcccccccagttatcggaacaggacggccagcagctgggaggaagactggtttgccaacatccccctggcatggaggcaacagctctataaactctacgaggccgactttgttctctttggctaccccaagccagaaaacctgctcagggactgagcccccagaagccctcacgctgcccccaacaaattgaatggctgtcccatgaggccgtcctttgaggatgggaccctgtggcctcctgggttctctcctggcttcctttgcttcctggtgtgacaggcagaggattccacgcccccccctcgcatctggagaccgtggtacagccaagaccgaagcacctcactctccagagttttgcgctccccacccccgcccttttgcaatctggatttgtttactccacagcctgtattcatggaacactgtgttaaatactgttttctaagattaatatatttcagatatatttaatacgaaagtgggaggaagctggagtaaagtgtggcgcccgcaaaaaaaaaaaaaaa

SEQ ID NO: 9 - protein, 419 aa, Mus musculus
MTKPRLFRLWLVLGSALMILLIIVYWDNVGTAHFYLHTSLSRPHILEPLPTQGLVEENVFTSDVDEFLDTLLSSDAKHNDLSRRKTEQPPAPAPSKPVLSHMEENVRGYDWSTHDAHQNPDRDRQQAERRSLLRDFCANASLAFPTKDRSFDDIPNYELNHLIVDDRHGVIYCYVPKVACTNWKRVMIVLSESLLDRGSPYRDPLDIPREHVHNTSTHLTFNKFWRRYGKFSRHLMKVKLKKYTKFLFVRDPFVRLISAFRSKFELENEEFYRKFAVPMLRLYANHTSLPASVSEAFSAGLKVSFANFIQYLLDPHTEKLAPFNEHWRQVYRLCHPCQIDYDFVGKLETLDEDAAQLLRFLKVDSQLHFPPSYRNRTASSWEEDWFANIPLAWRQQLYKLYEADFVLFGYPKPENLLRD

SEQ ID NO: 10 - DNA, 1728 bp, Mus musculus
  CDS (1)..(1116)
atgactgtcgcctgccacgcgtgccaggcacagcatgggaagacgctcctgttgcaggcggcccttgccggtggtggcaagtctgggtgctgcactcctgctcctgtgcgccctgcgtcccgggtaaccacaggaaaggatgcccaggacactgaatggcagggctccccaaaagcccttttgggggttccgacatttgaaaataaagctctgggctccagctggttcggtggagtgaggaagagtcccctacagctgttgcgtgacctggaccagggtccacgctccgcgatggccgaggtgcaccagcagcggcgtgagctgctgcgccgggcctgcagccgccacacgcgacgccaacgcctgctgcagccggaggacctgcgtcacgtgctggtggacgacgcgcaccggctgctgtactgctacgtgcctaaggtggcctgcaccaactggaagcgtgtgatgctggcgttgcgcggccgtggggatccaagcgcaatccctgcgcacgaggcgcatgcgcctggcctgctgccctcgctggccgactttgcgccggctgaggtcaactggcggctgcgcgactacctgacctttctcttcgtgcgggagcccttcgagcgcctggcgtcagcctaccgcaacaagctggcgcggccacacagcgcggccttccagcggcgctatggcacacgcatcgtgcgtcgcctacgaccacacgcgcagcccgatgcgctggcccgcggccacgacgtgcgcttcgccgagttcctggcctacctgctcgacccgcgcacgcgccgtcatgagcccttcaacgaacactgggagcgcgcacacgcgctgtgccatccgtgcctagtgcgctatgatgtagtgggcaagtttgagacgatagcagatgatgctgccttcgtgctggacctggtgggtgagcctgggctacgtttccctgctccaccgctgaggccagagaaggaccttacgcgtgagcaggcccggcgccttttccaggacatcagccccttctaccagcgtcgcctctttaacctctataagatggactttctgctcttcaattactctgccccttcctacctgcgactgcaataagggtgttgggtgcaatagagccagtggctgctgtgaccaggaggccaccaggaggtctggaacgaacctggttgtgtggattggagaccttatccagtgggcctgaccaagagtctggccactggtcacactcattccgactgggtagggtacaggttgctttaggtgaccataaccttgtcaggccgtttctgctgttagtttgatgtgtgtctcttcctcccactctgcagatgtcaggcttcttcctaggactccaggtttgtagttctttggtttggtttgagaggccatttctcagtcttgtctgtgtagaacctgtccgtggcatggtgctacaagacagaatgtcatggcttggttcagtgtggcctaaggtcttgtcagcatttactgcttaggagttaacatgagctgcctgccaccccagcagtcacaggatggtgagcactaccactccacatctacctggctgatctacctttgatctcagccttgcaagaggctggatcttcccctgtgtcagcaaaggccaagatgcaatactgtggcagcttttccagctcacttttattttttttgttgtttttttaaataaatatgttttgttac

SEQ ID NO: 11 - protein, 371 aa, Mus musculus
MTVACHACQAQHGKTLLLQAALAGGGKSGCCTPAPVRPASRVTTGKDAQDTEWQGSPKALLGVPTFENKALGSSWFGGVRKSPLQLLRDLDQGPRSAMAEVHQQRRELLRRACSRHTRRQRLLQPEDLRHVLVDDAHRLLYCYVPKVACTNWKRVMLALRGRGDPSAIPAHEAHAPGLLPSLADFAPAEVNWRLRDYLTFLFVREPFERLASAYRNKLARPHSAAFQRRYGTRIVRRLRPHAQPDALARGHDVRFAEFLAYLLDPRTRRHEPFNEHWERAHALCHPCLVRYDVVGKFETIADDAAFVLDLVGEPGLRFPAPPLRPEKDLTREQARRLFQDISPFYQRRLFNLYKMDFLLFNYSAPSYLRLQ

SEQ ID NO: 12 - DNA, 2073 bp, Mus musculus
  CDS (129)..(1259)
ccggccctggtccctgcctgcaccccgggagctggccacccactatccctcccctcccgagacctccagcccctgctgcagtcacctcccctgcagcctcgaggtcggcgaggtctggccgcagcaccatgtttccccgccctctgaccccactggctgccccgaaaagcgcggagaccctgggccgcacgccaaggcgggccccattgggccgggcccgggctgggctcggggggccgcccctgctgctgccgtccatgctgatgttcgctgtaatcgtggcctccagcggactgctgctcatgatcgagcgaggcatcctatcggagatgaaaccccttcccctgcaccctcccagccacaaaggcgcggcctggagcgggacagatcctaagcctagaggcctatccttggatgctggggactcggacttgcaagtgagggaggacatccgaaaccggaccttgagggccgtgtgcggacaaccaggcatgccccgggacccctgggacttgccggtgggacagcggcgcaccctgctgcgccacattctcgtaagtgaccgctaccgcttcctctactgctatgtccccaaagtggcctgctctaactggaaacgtgtgctgaaggtgctggctggcgtcctgaacaacgtggatgtccgcctcaagatggaccaccccagtgacttggtgtttctggcagacctgcggcctgaggagattcgctaccgtctgcagcactacttcaagttcctgtttgtgcgagaccccttggaacgcctcctgtctgcttaccgtaacaagtttggagagatccgagagtaccagcagcgatatggggccgaaattgtcaggcgctacagggctggagctggtcccagccctgcaggggacgatgtcaccttcccagagttcctgagatacctggtggatgaggatcctgaacatatgaatgagcattggatgcctgtgtaccacctgtgccaaccatgtgctgtgcactacgacttcgtgggttcctatgagaggctggaggctgatgccaaccaggtgctggagtgggtgcgggccccaccccatgtccggttcccagctcgccaggcctggtaccggccagccagcccagaaagtctgcattaccacttgtgcaatgttccacgggccctgcttcaagatgtgctacctaagtatatcctggacttctccctctttgcttacccactgcccaatgtcaccaaggaagcctgtcaccaatgacagtaggccagcaccttttggagtttgggtttaatgatatcagctttgggatgtctttcagagaaactcctggctctgggtggcttcctggtttctctaggtgtctccatatctcagtggtaaggactgtccttggaggtccttgtccacagtggctcagaggacagagctagaaaggaggcctgctgctttcactggtgaactgcctctcttaggggcctgtggtatccgtgtctgcagggcaccagtggttattaaagccatatgtttgatcgaaagactgacttcagccccctggctgctgggtctatgcagtccacctggtctgttgtaatttaacctgtggccaaatcccaaatatgacactagccaagcacatgatcatgcctaggaccaatggctgtgaccccctattcacccatcccatggacctcaggactggagtgagctgtggtgccttagaaatgaaatgtgtgcaattctactccagacttttacatttcctcctcttgctaggtctgaatcatttttctaaggaaagagaaacggaagtggggcccttacctcgaagctctaaagcccagcccctcaagcatccaaagacgcctgtgcctgacctcttcctagggctcctggagcatcttcaataagcctcccttccctacaaacctttggagactatgtgagactgtatggcccatatatctggctgtcacttgtctaatgcatttatttaaaatgtgtatattttaataggatccttgtaagggctgacttttaataaagctttttcatatacaaaaaaaaaaaaaaa

SEQ ID NO: 13 - protein, 376 aa, Mus musculus
MFPRPLTPLAAPKSAETLGRTPRRAPLGRARAGLGGPPLLLPSMLMFAVIVASSGLLLMIERGILSEMKPLPLHPPSHKGAAWSGTDPKPRGLSLDAGDSDLQVREDIRNRTLRAVCGQPGMPRDPWDLPVGQRRTLLRHILVSDRYRFLYCYVPKVACSNWKRVLKVLAGVLNNVDVRLKMDHPSDLVFLADLRPEEIRYRLQHYFKFLFVRDPLERLLSAYRNKFGEIREYQQRYGAEIVRRYRAGAGPSPAGDDVTFPEFLRYLVDEDPEHMNEHWMPVYHLCQPCAVHYDFVGSYERLEADANQVLEWVRAPPHVRFPARQAWYRPASPESLHYHLCNVPRALLQDVLPKYILDFSLFAYPLPNVTKEACHQ

SEQ ID NO: 14 - DNA, 6000 bp, Mus musculus
  CDS (496)..(1914)
cttagccactgaaccatctctccagcctctgttttggggtgtttgtttgagacagaatcaaaaggctggtctaaagtacatattgtagctaaagatggcttccaactcctgccttgcctccagagtgttagggtgtgacctttaaatgacctattaaagaaaccccaacaggtgtagagtacacctgtgatcccagctcttaggaggttggacagatggataaagaggtccaggtgtcccggactacatagagagaccctatctcaaaagagaggcgaagacttaggttttgagagtgggcctgaggtctctcttcaaaagttttatagaaagatgtctctgttccctgtctatgaacacggatggcctgagcacctgtctcttcacaggatcagagtgtcccccacctgaagagggctgattgggtcccaagctatgctcctgagctgagtgcctgcagccagtctgaggaactccatggcgccccctctccccatggagaaaggactcgctttgcctcaggatttccgggaccttgtacacagcctaaagattcgaggcagatacgtcttgttcctggcatttgtggtcatagtttttatcttcattgaaaaggaaaataaaatcatatccagggtctccgacaagctgaagcagatccctcattttgtggcagatgccaacagcactgacccagccctgctcttatcggagaatgcatctctcttgtccctgagcgagttggattccaccttttcccatctgcggagccgcctgcacaacctgagcctgcagctgggcgtggagccagcaatggagagccaggaggctggggcagagaagccatcccagcaggctggagcagggacccggcgccacgtgcttctcatggccaccacccgcacgggttcctcgttcgtgggcgagttcttcaaccagcagggcaatatcttctacctcttcgagccactgtggcacatcgagcgcaccgtgttcttccagcagcgaggcgccagcgcggctggttcagccttggtctaccgtgatgtcctcaagcagttgttgctatgcgacctgtatgtgctggagcccttcatcagccctccgcccgaggaccacttgactcagttcctgttccgccggggatccagccgttcactctgcgaggatccggtgtgcacacccttcgtcaagaaggtctttgagaagtaccactgcaggaaccgtcgctgcgggccactcaacgtgaccttggcgggcgaggcctgccgccgcaaggaccacgtggccctcaaggctgtgcgcatccgtcagctggagttcctgcagccgctagttgaggacccgaggttggatctacgagtcattcagctggtgcgcgacccccgggccgtgctggcttcacgcatagtggcctttgcgggcaagtatgagaactggaagaagtggctgtccgaggggcaggaccagctgagcgaggatgaggtgcagcgattgcggggcaactgtgagagcatccgcctgtctgcagagctgggcttgcggcagccagcctggctgcgcggtcgttacatgctggtgcgctatgaggatgtggcacgcaggccactgcagaaggcccgagagatgtacagctttgcgggcatccccttgaccccgcaggtggaggactggatccagaagaacacgcaggcgacacgcgacagcagcgatgtctactccactcagaaaaactcttctgagcagtttgagaagtggcgcttcagcatgcctttcaagctggcacaggtggtacaggctgcctgtggcccgaccatgcacctctttggctacaagttggccagggatgccgcctcactcaccaaccgctccatcagcctgctggaggagcggggcaccttctgggtcacgtagtgggggatgtctgggacccttggaactccttcttgtgaaaggctggccctgcttccctcacacccagcctggcagtgagacatagccctggcagaaagtcaaaatggggagcgatgatgggaacatagcccctggctgtagcggtagggccccctgccagctagactccccagagcagctacagctagggccttgggctcctctgaggacaccctgtctccttagtggtactggtcataaggtgtcctcaccctatgacctgcagtgtcccgagcaggtcaaggtaggttcctgtgtgtggacacacctccctagctctttctcacacagtctacacgaagcctgtaaaggcctgtaggttgtgtgggctggagtccaagtatttaacaaccagaaggggtgtagaccctctgcagcctctcagacctcctactgtattaagtgttaacctcttccgctctgagtcagagaagctgggatctggctgagtcctgggaaggaggaggacagcctagggtgaggaaggggacctttgaagctcctcagggaacagtggctgtgtaccagctcatagaaaatggtttgatcagctgttctagtcactcatgagtatcaatcagcctgtgtagagcaagacacacaaagtgcattgaaaacagacaaggccaggggtgtggctcagcggtaaagcccttgcctctctcatgcccagggccctaggtgtgattcttagcactataaatataagggaaaataagccatacatacgtgtgcagtacagagagagacagaaaagcgtaataaacattcccccctctcataagcacacgctctgcctctgtctctgtctctgtctctctctgtctctgtctctctctgtctctctctctcactctctctctctctctctctctctcacacacacacacacacacacacacacaaacacacacacacacactggtacagaaaagcttcccttctccactctttatgctcaccatgtttttaggatttttgtttgtttgttttgttttgggtttctatatatctaaacaaggagccttaaattacatctttttgggattacgtggcgagggggagcagcagggagcatttgcttctggtaaaaggatagaccagaaaggacttccccttggatgatcggagtcatgcagagcccccagggtcccacatgttctgtgtgaacttcatgtggaatgactcacagaagtgactaccttaggcgctcgctctgtagctcaatgtgcgtagagtttgtctattgtataggaagccctgggttctgtgccctgccccacaccatataggtatgatggcgtgtacccatatcccagcattcaggaaatcaaaggttggcggtcaaaagttcaaggtgcagctatgtatcttttgagatgtccgagtctataagctccctctactgagagctgctagtattccttctcaagaacaggttatttgaaaatctcttcttgtaagccccaacatttgggggaggggaggatgggggaactcttgactgagcagctaggtttccccaagcagaagttcttctctcccagtgcaagctgaggtttagtgccccggctagcctcggaactggctcagtgggggttggcacgctgacttcctggacaattgctgcatctgacactgtgagcgcccaggacaccggatgtgtagcatggatgtgggcctagcacaggtgtggaagaggacagtcaggacactcactgttggtgtttgttatccacctgttcagccgccgggtcccacacataggtcatctttcgtcactcaagccggcctctgtttttgattttaacaatccaagagcaagtgtgtaggggacaaagagacaccagctcttcatacttgatggagaccgggacaggatgctgcaggcaggctcgggagtgcattatcgtttcttctgagctcttcatccaggccatattcccttttctgcatcgcatctggggtgggaggggctgagctgggagtttccgtccttcttccctgtgggggtgggagatggggctcaaggtctccatctctcggctccctgaggacagaacccccacagtggacctttgggccttctcaggacattgacaatgttgtgtgcactgcaagttgactttatttattttgtaggaaaaagagatggtattctttagcaggatctgaaactgtaccctagtcaagaagtacaattaataacattattattaataacaattgggatgattcaaaggtcacacacacaccagaccacccaagaaccatgtaggagatgaggcggagccaggtcatggaagcccagaatgctacagagattctgtgggtctattattgatcagaaaatacaacatgggggggccttttctatggcataactcaggtgtctgcaaagacagagcagctcaggtgggtggataggcaggcagatggagccttgaatcacatcccctgaggctcagccagccagtgcgaatcctcaaggttcggaaagggacagtgtagcggcaaactactgggcatcttctctgatgcttagaggctcttaccaaggagcttgatggagaaagtggccatgttggtggcatgggacaactgctcacccaacttcaaagatcaaagggcacccaggtggcctatgacagtgacactctttcctaccattaggggtgtctgcccccactgaaagccatgaaatttctggccctaagggggtaggaaggacttaggagtagcagatggtttgatcccatcccccccacacacacacacacatccctcagctgtcttccacattagagccacttcagttgtccatggacttgtccctttgagacatcctggattttgaaggatagaaacatccccaagatggtctcgtgttaatcccacaacagaggcagaagggtcatactgagagagagagagagagagagagagagagagagaggagtgggggccagaccctcaagaagccaagtgggtctggtcaacctgtgcacatgagaaggagggaacatcactaaaatcagggcctgggctggtgtgttgttggtgagatcccgtggagtggctggctagatatggatgagttttctgagcatgctcacacacccccaacttcacattcttagaaatagcacaaccataatgccttacctcaaaaggatgaggcaaagcttgcaattaattcccagtgtctgaagacctccgggatcctttgagctgtgtgtccttgtcagtacatggggacaggctccttaggtattcctgacatagaggtaaggtgctgcccttgctgccttgcataagctgtgacaagcttcttactgggcacatagaacggctctgtcatctgcttccactaaatttgggcttggactttgcctcctgccaaatctccatctctgctggatagtctagtccctagggtctaaccaccaccctccacttcctggtgggtcctacaagcgctgtctttgtgccagtacccggatggtgtcctgcctcatggctaaatggtacaggacatcttcccagactgagtggtcatggcatgtgcatgtatgttcatgagtacatgcatggtgtgtgggggtggatgggtgcattctgttctgcttctggtgcagctacacagccacaacctctttctgtcattgaccttcttggtcttcttgtagccacagataatcttccaatgcccgattctgctgttctcatctgagagctgacaacccagcgctcagagtagagttcatgacctaggaaacccttctcctggtagcttactgaacttatttaattaaaaacgaacatataggggttggagagatggttcattggttaagagcaccggctgcttttgcaaaggacctgagttcaaatcccagcaaccatatggtggcttacaaccatctgtaatgagttctggtgccctcttctggcatgcaggtgtacatgcagatagagcactcctatgcataaaataaataaatcttttaaataaataaataaatgaacatgaaaaaaaaaaaaaaa

SEQ ID NO: 15 - protein, 472 aa, Mus musculus
MEKGLALPQDFRDLVHSLKIRGRYVLFLAFVVIVFIFIEKENKIISRVSDKLKQIPHFVADANSTDPALLLSENASLLSLSELDSTFSHLRSRLHNLSLQLGVEPAMESQEAGAEKPSQQAGAGTRRHVLLMATTRTGSSFVGEFFNQQGNIFYLFEPLWHIERTVFFQQRGASAAGSALVYRDVLKQLLLCDLYVLEPFISPPPEDHLTQFLFRRGSSRSLCEDPVCTPFVKKVFEKYHCRNRRCGPLNVTLAGEACRRKDHVALKAVRIRQLEFLQPLVEDPRLDLRVIQLVRDPRAVLASRIVAFAGKYENWKKWLSEGQDQLSEDEVQRLRGNCESIRLSAELGLRQPAWLRGRYMLVRYEDVARRPLQKAREMYSFAGIPLTPQVEDWIQKNTQATRDSSDVYSTQKNSSEQFEKWRFSMPFKLAQVVQAACGPTMHLFGYKLARDAASLTNRSISLLEERGTFWVT

SEQ ID NO: 16 - DNA, 2080 bp, Mus musculus
  CDS (147)..(1601)
caccgcccggctgctccactccgctccacccaacattgagggagacccgaagaggccggagccgaggactttgggctgggttttctggacagaaccagcaggcgcctactctgctctgggtggggagagtgaggattcggtgaactatgaagggccggcggcggcggcgccgaaagtattgcaagttcacgctgctcttggcgctgtacacgcttttgctacttcttgtcccctctgtactggacagccacagcgagcaggacaagggcaggaactgccccggcctgcagcgcagcttgggtgtgtggagcctggaggcggcggcggccggggaacgtgagcagggcgctgaggtgcggtccctggccgaaggaaacccggatcgatcccccgggtcccccggcaacctcagcgccgtcggtgaggcggtgacccaggaaaagcaacacatctatgtgcatgccacctggcgcaccggctcgtccttcttgggcgaactcttcaaccagcacccggacgttttctacttgtacgaccccatgtggcatctgtggcaggcactgtatccgggcgacgcggagagcctgcagggcgcactaagagacatgctgcgctccctcttccgctgtgatttctctgtgctgcgcctgtacgcgcagcctggggaccctggggagcgagcaccggactcggccaacctcaccacggccatgcttttccgctggcggaccaacaaggtcatctgctcgccgcctctgtgccccgccgcgccccgggcacgcgcggacgtgggactcgtcgaggacaaagcctgcgaaagtacctgcccgcccgtttcgctccgcgccctggaggccgagtgccgcaagtacccggtggtggtcatcaaagacgtgcggctactggacctgggagtgctggtccctctgctgcgtgacccaggcctcaacctaaaggtggtgcaactcttccgagaccctcgggccgtgcacaactcgcgcctcaagtcgaggcagggactgctgcgcgaaagcatccaggtgctgcgcacgcgccagaggggcgaccacttccaccgggtgctgctggcgcatggagtggatgcccgtccgggaggccaggcccgggctctgccctcggcgccacgcgctgatttcttcttaaccagcgcgcttgaggtgatctgtgaagcgtggcttcgcgacctgctattcacccgcggcgcgcccgcctggctgaggcgtcgctacctgcggctgcgttatgaggacctggtgtggcagccccaagcccagctgcgccgcctgctgcgcttctctgggttgcggacactcgccgcgcttgatgccttcgcattcaatatgacgcggggctcggcctacggcgccgatcgtcccttccacttgtctgcgcgggacgcccgagaggctgtgcacgcctggcgcgaacgtctgagccaagagcaggtgcgccaagtggaaaccgcctgcgcccctgccatgcgtctgcttgcctaccctcgaagtggggacgaacgcgacaggaagaccgtcagggaaggggagacaccactggagaccaaggccaattgggctgtgtaataccctgatccctgaaccctgccccggggcgtattcaggtcagtggccataaaaaggtgaactcagcatgctgcccccgcactggagaggctgcacggtggaggcgatctatcacactgtgagacactgggactgatttggtatcaactgctgtgccattctcctggtcaggagcatcacaagctgttaagtaatgacagacaccttggctgagatgaagtttccagaaaggaagtaacagtgcaatgtggatatttgtgaccacaacataggaaaagctgtacttcccaggctgaacttggctcagcttgagccatttcaacaaggcatcctcacaataatgaagagatgtgatctggtttcctttcacatcagccaagatgtctggacaaaaccatcaatgtgaataagggccaagtgcagttgtgtctctcttgattaaattacttcatattaaataaaaaaaaaaaaaaaaaaaa

SEQ ID NO: 17 - protein, 484 aa, Mus musculus
MKGRRRRRRKYCKFTLLLALYTLLLLLVPSVLDSHSEQDKGRNCPGLQRSLGVWSLEAAAAGEREQGAEVRSLAEGNPDRSPGSPGNLSAVGEAVTQEKQHIYVHATWRTGSSFLGELFNQHPDVFYLYDPMWHLWQALYPGDAESLQGALRDMLRSLFRCDFSVLRLYAQPGDPGERAPDSANLTTAMLFRWRTNKVICSPPLCPAAPRARADVGLVEDKACESTCPPVSLRALEAECRKYPVVVIKDVRLLDLGVLVPLLRDPGLNLKVVQLFRDPRAVHNSRLKSRQGLLRESIQVLRTRQRGDHFHRVLLAHGVDARPGGQARALPSAPRADFFLTSALEVICEAWLRDLLFTRGAPAWLRRRYLRLRYEDLVWQPQAQLRRLLRFSGLRTLAALDAFAFNMTRGSAYGADRPFHLSARDAREAVHAWRERLSQEQVRQVETACAPAMRLLAYPRSGDERDRKTVREGETPLETKANWAV

SEQ ID NO: 18 - DNA, 4713 bp, Homo sapiens
  CDS (514)..(2199)
ggaaatctggcattttttaaagtttgcgccccacaaagaggaaatattccaaaggtactcaggatgtaaaaggggagatcttcacagatgcctccgtggatggcatggcaatccatccatcaatgagaagaccatgatttcttttaattttctgtgtgtttccacattccccagtgagaattcttccacctttttttgtgccatgggaaaaacctgaagggcaggcagagctgctcccgaacttgtgaccttctctgaggttgcagcggctcttgtagaacatgactctgggacatcacttccttttgttttctttcggagctgaaccaaagaatgtgcaccctctttctctagtgctgtggtgtctgcttatttttgtatttgtgctttccatccatcttctgtgatcacaaggcattcttaaggttttctagcacgacttgcggacatccagactcgtggggggcccacccatggctcggtaagccagcagcccagggcactggcactaccatgaggcactgcattaattgctgcatacagctgttacccgacggcgcacacaagcagcaggtcaactgccaagggggcccccatcacggtcaccaggcgtgccccacgtgcaaaggagaaaacaaaattctgtttcgtgtggacagtaagcagatgaacttgcttgctgttctcgaagtgaggactgaagggaacgaaaactggggtgggtttttgcgcttcaaaaaggggaagcgatgtagcctcgtttttggactgataataatgaccttggtaatggcttcttacatcctttctggggcccaccaagagcttctgatctcatcacctttccattacggaggcttccccagcaaccccagcttgatggacagcgaaaacccaagtgacacaaaggagcatcaccaccaatcctctgtaaataatatttcatacatgaaggactatccaagcattaaattaattatcaacagcatcacaactaggattgagttcacgaccagacagctcccagacttagaagaccttaagaagcaggagttgcatatgttttcagtcatccccaacaaattccttccaaacagtaagagcccctgttggtacgaggagttctcggggcagaacaccaccgacccctacctcaccaactcctacgtgctctactccaagcgcttccgctccaccttcgacgccctgcgcaaggccttctggggccacctggcgcacgcgcacgggaagcacttccgcctgcgctgcctgccgcacttctacatcatagggcagcccaagtgcgggaccacagacctctatgaccgcctgcggctgcaccctgaggtcaagttctccgccatcaaggagccacactggtggacccggaagcgctttggaatcgtccgcctaagagatgggctgcgagaccgctatcccgtggaagattatctggacctctttgacctggccgcacaccagatccatcaaggactgcaggccagctctgcaaaggagcagagcaagatgaatacaatcattatcggggaggccagtgcctccacgatgtgggataataatgcctggacgttcttctacgacaacagcacggatggcgagccaccgtttctgacgcaggacttcatccacgcctttcagccaaatgccagactgattgtcatgctcagggaccctgtggagaggttgtactcagactatctctactttgcaagttcgaataaatccgcggacgacttccatgagaaagtgacagaagcactgcagctgtttgaaaattgcatgcttgattattcactgcgcgcctgcgtctacaacaacaccctcaacaacgccatgcctgtgaggctccaggttgggctctatgctgtgtaccttctggactggctcagcgtttttgacaagcaacagtttctcattcttcgcctggaagatcatgcatccaacgtcaagtacaccatgcacaaggtcttccagtttctgaacctagggcccttaagtgagaagcaggaggctttgatgaccaagagccccgcatccaatgcacggcgtcccgaggaccggaacctggggcccatgtggcccatcacacagaagattctgcgggatttctacaggcccttcaacgctaggctggcgcaggtcctcgcggatgaggcgtttgcgtggaagacgacgtgagagctgaattgttgctgcacgtgctgggcccgccaatgccgtcatcatcaggattttacaaatctctttgcggggaactgtttcactcatggtatggaaaaccccaggactctgccactctaggcacacatgaattataaccattttggaatttccttcgtgatgttcgagagctcagcaatggacccctcacagagctcctctatccgaggccattggagaccccagtttctcaagaattcagctctgctctgagcgtcctggagcttggggatgcagccagctggcctgcactgggtgtggagagaacacctagggaaggcagcctggccctgcccgcctccgccttctggagagcctctgggttctgagtcagcaagccagaggtcatgccacaggcctggctggaacttacacttcacgttccctttttttccccctagagatggggtctcgccgtgttgcacagactgtctgtattcaatggctatcttcacaggtgtgatcataccacattcacttctgaaacactcttgttgcgatcgctaacctcactgggacagagaaccgcagtctttcgagaatggaggctcttcattttttttttctcctttactccaaactcagccctccagtttcttcagatgtaaaccctgttaacgtcactgtttccaaaaggaaaaaaataagtcagtttttggcagcaccttcatctttctgacctcctcctattctgtccttgtggacttatgtttaacatagaaaatgaatgcgtttaaaacaaaaccactttctgcatttaaccagtcctggctctctctctgctgcctcttcatacgttttctcaagaacttcagtttataattggaagagaaatttttgctgttaatgccagaatgagcaacctcaaggaattgaacacttcttggaaaatctaggtaattcaagccctcatcaggtttacaagatcatcagagaaacagaggattttaatttttagttctggccggctacaggctccatttctctgccttcccattggaaatagtttatttccacattctccactgcgtgtggtcaaagttcctcacccagcaagggactatagatactcgtgtcccaattccaaaacacaatgcacaagctgaacttgggctgaacgtggcgtgttgagatttggaatgaggtttctaagagccgtgttcttcatggaattttccaggccacttggcagcttggtttaccgatggatgggctagagatcttgtcgtttcttggaagtcacagggaagattgaagagaacgcttgagcatccttggcaacagcccaggtgggacctggatgaagctttgcactcaagtattgtcaagggaagcttcctgtgaaccaaagttctcaggccaaggtctcgcccaccaaagccagaaagtgcaagcacccgtctacccagctctaacttgtatgtgtgagacagaccaggcttcgggggtaggaggatctgcagttgttcagccgtctttctgctggtgttgtctttctgccatcagagaagggacacacagcccgttcgaaggtgtgcagagggctctgagcgccaggatggccagggctgtttttgctactgaaggagcgtgtgtcctgaactcccacttgcagggacagtccccaccttctctatagccggcactgggagcagccgccagcagggaaatctggcctgagcacaaggatgctttagggagagatcacttcagtgtgtgtgtatatttatttgcagtacagtgcgcgcgtgtgtgtgtgtgtacgcgcacgtgtgggtgagtgcgtcttctgagtgggttctgttcagttgctaatgaggctcctccgctctggacacaacccttttatagattaatttctctgccaattaacttgtcattttcagtacatattttactattccacaccaaccataattacaacaagggatttttcttatgcactcctatgcatgtgaataacatgtggtgtaattctgcttcttacagaagtattactgaaggtattatttccaatattatttggtttattatgcggatcttttttatatatgcagtcccatcccttctgtgccactcaatgccatccagacatggtttttccctccaggggcctttctctccagagggcacttcggctgcctctgcttcctctcattcgaggcccggctcttgctgacagaataggttccgttctgggcggtggttctcgagcctgccattcaaaaccaaagcaaattggagcatttctcacaacatggtattgaagttcctttttgttctcaaaagttgtgaccgtgttaaattgtactcccttagtcctgtaaggtatgttaagtgaatcgcagttacgctgtacttttattaatatttaacataattaaagatggacccataagagtgacgcctgtggagcgcgtgctcttcctctgcagccaaaaaaaaaaaaaaaaaaaaaaaaaaaaaaaaaaa

SEQ ID NO: 19 - protein, 561 aa, Homo sapiens
MRHCINCCIQLLPDGAHKQQVNCQGGPHHGHQACPTCKGENKILFRVDSKQMNLLAVLEVRTEGNENWGGFLRFKKGKRCSLVFGLIIMTLVMASYILSGAHQELLISSPFHYGGFPSNPSLMDSENPSDTKEHHHQSSVNNISYMKDYPSIKLIINSITTRIEFTTRQLPDLEDLKKQELHMFSVIPNKFLPNSKSPCWYEEFSGQNTTDPYLTNSYVLYSKRFRSTFDALRKAFWGHLAHAHGKHFRLRCLPHFYIIGQPKCGTTDLYDRLRLHPEVKFSAIKEPHWWTRKRFGIVRLRDGLRDRYPVEDYLDLFDLAAHQIHQGLQASSAKEQSKMNTIIIGEASASTMWDNNAWTFFYDNSTDGEPPFLTQDFIHAFQPNARLIVMLRDPVERLYSDYLYFASSNKSADDFHEKVTEALQLFENCMLDYSLRACVYNNTLNNAMPVRLQVGLYAVYLLDWLSVFDKQQFLILRLEDHASNVKYTMHKVFQFLNLGPLSEKQEALMTKSPASNARRPEDRNLGPMWPITQKILRDFYRPFNARLAQVLADEAFAWKTT

SEQ ID NO: 20 - DNA, 536 bp, Mus musculus
acaaagccatgaagccggcgctgctggaagtgatgaggatgaacagaatttgccggatggtgctggccacttgcttcggatcctttatcttggtcatcttctatttccaaagtatgttgcacccagtcatgcggaggaaccccttcggtgtggacatctgctgccggaagggatcgagaagtcccctgcaggagctctacaatcccatccagctggagctatccaacactgccatcctgcaccagatgagacgggaccaggtgacagacacctgccgggccaacagtgccatgagccgcaagcgcagggtgctgacccccaacgacctgaagcacctggtggtggatgaggaccacgaactcatctactgctatgtgcccaaggtagcgtgcaccaactggaagaggctcatgatggtcctgagtggccggggcaagtacagcgatcccatggagatcccagccaacgaagcccacgtgtcggccaacctgaagacccttaaccagtacagcatcccagagatcaaccaccgcttg

SEQ ID NO: 21 - DNA, 660 bp, Mus musculus
gccaggagtgggcccagcccagggcagcatgaccaagccgcggctcttccggctgtggctggtactagggtcggctctcatgatccttttgatcattgtatattgggacaacgtgggaaccgcccacttctatctgcacacgtctctctccaggccacacatcctagaaccccttcccacccagggattggtggaggagaacgtgttcacatctgacgtggatgagtttttggatactctccttagttctgacgcgaagcacaacgacctttccaggagaaaaactgagcagcccccggcgcccgcccccagcaagccagtcttgagccacatggaggagaacgtgagaggctacgactggtccactcatgatgcccatcagaaccctgaccgggacaggcagcaggccgagaggaggagcctgctgagagacttctgtgccaacgccagcctggcattccccaccaaggaccgctcttttgacgacatccccaactacgaactgaaccacctgatcgtggacgaccgccacggggtcatctactgctacgtgcccaaggtggcctgcaccaactggaagcgagtgatgatcgtgctgagcgagagcctgctggaccggggcagcccctaccgagaccccctggacatcccccgggaaca

SEQ ID NO: 22 - DNA, 600 bp, Mus musculus
atgactgtcgcctgccacgcgtgccaggcacagcatgggaagacgctcctgttgcaggcggcccttgccggtggtggcaagtctgggtgctgcactcctgctcctgtgcgccctgcgtcccgggtaaccacaggaaaggatgcccaggacactgaatggcagggctccccaaaagcccttttgggggttccgacatttgaaaataaagctctgggctccagctggttcggtggagtgaggaagagtcccctacagctgttgcgtgacctggaccagatgtttggcagctgtgagctatgggtagtcagtggggagcggcagaaagtgggtccacgctccgcgatggccgaggtgcaccagcagcggcgtgagctgctgcgccgggcctgcagccgccacacgcgacgccaacgcctgctgcagccggaggacctgcgtcacgtgctggtggacgacgcgcaccggctgctgtactgctacgtgcctaaggtggcctgcaccaactggaagcgtgtgatgctggcgttgcgcggccgtggggatccaagcgcaatccctgcgcacgaggcgcatgcgcctggcctgctgccctcgctggcc

SEQ ID NO: 23 - DNA, 600 bp, Mus musculus
gcgccccctctccccatggagaaaggactcgctttgcctcaggatttccgggaccttgtacacagcctaaagattcgaggcagatacgtcttgttcctggcatttgtggtcatagtttttatcttcattgaaaaggaaaataaaatcatatccagggtctccgacaagctgaagcagatccctcattttgtggcagatgccaacagcactgacccagccctgctcttatcggagaatgcatctctcttgtccctgagcgagttggattccaccttttcccatctgcggagccgcctgcacaacctgagcctgcagctgggcgtggagccagcaatggagagccaggaggctggggcagagaagccatcccagcaggctggagcagggacccggcgccacgtgcttctcatggccaccacccgcacgggttcctcgttcgtgggcgagttcttcaaccagcagggcaatatcttctacctcttcgagccactgtggcacatcgagcgcaccgtgttcttccagcagcgaggcgccagcgcggctggttcagccttggtctaccgtgatgtcctcaagcagttgttgctatgcgacctgtat

SEQ ID NO: 24 - DNA, 720 bp, Mus musculus
tggggagagtgaggattcggtgaactatgaagggccggcggcggcggcgccgagagtattgcaagttcacgctgctcttggcgctgtacacgcttttgctacttcttgtcccctctgtactggacagccacagcgagcaggacaagggcaggaactgccccggcctgcagcgcagcttgggtgtgtggagcctggaggcggcggcggccggggaacgtgagcagggcgctgaggtgcggtccctggccgaaggaaacccggatcgatcccccgggtcccccggcaacctcagcgccgtcggtgaggcggtgacccaggaaaagcaacacatctatgtgcatgccacctggcgcaccggctcgtccttcttgggcgaactcttcaaccagcacccggacgttttctacttgtacgagcccatgtggcatctgtggcaggcactgtatccgggcgacgcggagagcctgcagggcgcactaagagacatgctgcgctccctcttccgctgtgatttctctgtgctgcgcctgtacgcgcagcctggggaccctggggagcgagcaccggactcggccaacctcaccacggccatgcttttccgctggcggaccaacaaggtcatctgctcgccgcctctgtgccccgccgcgccccgggcacgcgcggacgtgggactcgtcgaggacaaagcctgcgaaagtacctgcccgcccgtttcgc

SEQ ID NO: 25 - RNA, 27 nt, Artificial
  an artificially synthesized sequence
ggagcagagcaagaugaauacaaucag

SEQ ID NO: 26 - RNA, 27 nt, Artificial
  an artificially synthesized sequence
gauuguauucaucuugcucugcuccau

SEQ ID NO: 27 - DNA, 20 bp, Artificial
  an artificially synthesized primer sequence
gtgagttctgctgcggtcca

SEQ ID NO: 28 - DNA, 21 bp, Artificial
  an artificially synthesized primer sequence
agtccatgctgatgcccagag

SEQ ID NO: 29 - DNA, 19 bp, Artificial
  an artificially synthesized primer sequence
acccgatggcaacaatgga

SEQ ID NO: 30 - DNA, 20 bp, Artificial
  an artificially synthesized primer sequence
accagcagggccttgttcac

SEQ ID NO: 31 - DNA, 25 bp, Artificial
  an artificially synthesized primer sequence
catccgtaaagacctctatgccaac

SEQ ID NO: 32 - DNA, 19 bp, Artificial
  an artificially synthesized primer sequence
atggagccaccgatccaca

SEQ ID NO: 33 - DNA, 23 bp, Artificial
  an artificially synthesized primer sequence
ttctggccaacggtctagacaac

SEQ ID NO: 34 - DNA, 21 bp, Artificial
  an artificially synthesized primer sequence
ccagtggtcttggtgtgctga

SEQ ID NO: 35 - DNA, 25 bp, Artificial
  an artificially synthesized sequence
acccccaactcggaacgatgcggct

SEQ ID NO: 36 - DNA, 24 bp, Artificial
  an artificially synthesized sequence
tgcatgttctcgtccatcctgctg

SEQ ID NO: 37 - DNA, 26 bp, Artificial
  an artificially synthesized sequence
cgccaccgtgtactgtactgtgaagt

SEQ ID NO: 38 - DNA, 25 bp, Artificial
  an artificially synthesized sequence
aggctgctccaactggaagagggtg

SEQ ID NO: 39 - DNA, 24 bp, Artificial
  an artificially synthesized sequence
atatagtatctaggatatatgtag

SEQ ID NO: 40 - DNA, 25 bp, Artificial
  an artificially synthesized sequence
gaagtaccaaaagctggctgctcta

SEQ ID NO: 41 - DNA, 26 bp, Artificial
  an artificially synthesized sequence
ttctatcacttggactatttgatgtt

SEQ ID NO: 42 - DNA, 25 bp, Artificial
  an artificially synthesized sequence
tacacaactccacatttgtaatttg

SEQ ID NO: 43 - DNA, 24 bp, Artificial
  an artificially synthesized sequence
ccagaagccaagctcattgttatg

SEQ ID NO: 44 - DNA, 25 bp, Artificial
  an artificially synthesized sequence
ctgtggagaggttgtactcagacta

SEQ ID NO: 45 - DNA, 26 bp, Artificial
  an artificially synthesized sequence
atttgcctggaagacaacgtgagagc

SEQ ID NO: 46 - DNA, 27 bp, Artificial
  an artificially synthesized sequence
gtcccttctgcagaagctgggcccact

SEQ ID NO: 47 - DNA, 25 bp, Artificial
  an artificially synthesized sequence
gcgccccctctccccatggagaaag

SEQ ID NO: 48 - DNA, 25 bp, Artificial
  an artificially synthesized sequence
gctttgcctcaggatttccgggacc

SEQ ID NO: 49 - DNA, 27 bp, Artificial
  an artificially synthesized sequence
ggttcagccttggtctaccgtgatgtc

SEQ ID NO: 50 - DNA, 25 bp, Artificial
  an artificially synthesized sequence
gcagttgttgctatgcgacctgtat

SEQ ID NO: 51 - DNA, 23 bp, Artificial
  an artificially synthesized primer sequence
tgttcctggcatttgtggtcata

SEQ ID NO: 52 - DNA, 21 bp, Artificial
  an artificially synthesized primer sequence
ccaactcgctcagggacaaga

SEQ ID NO: 53 - DNA, 25 bp, Artificial
  an artificially synthesized primer sequence
gtgtggagcaacatgtggaactcta

SEQ ID NO: 54 - DNA, 20 bp, Artificial
  an artificially synthesized primer sequence
ttggttcagccactgccgta

SEQ ID NO: 55 - DNA, 50 bp, Artificial
  an artificially synthesized sequence
acaaagccatgaagccggcgctgctggaagtgatgaggatgaacagaatt

SEQ ID NO: 56 - DNA, 26 bp, Artificial
  an artificially synthesized sequence
caacctgaagacccttaaccagtaca

SEQ ID NO: 57 - DNA, 26 bp, Artificial
  an artificially synthesized sequence
gcatcccagagatcaaccaccgcttg

SEQ ID NO: 58 - DNA, 25 bp, Artificial
  an artificially synthesized sequence
gccaggagtgggcccagcccagggc

SEQ ID NO: 59 - DNA, 27 bp, Artificial
  an artificially synthesized sequence
atgaccaagccgcggctcttccggctg

SEQ ID NO: 60 - DNA, 28 bp, Artificial
  an artificially synthesized sequence
agagcctgctggaccggggcagccccta

SEQ ID NO: 61 - DNA, 28 bp, Artificial
  an artificially synthesized sequence
gagaccccctggacatcccccgggaaca

SEQ ID NO: 62 - DNA, 26 bp, Artificial
  an artificially synthesized sequence
atgactgtcgcctgccacgcgtgcca

SEQ ID NO: 63 - DNA, 26 bp, Artificial
  an artificially synthesized sequence
cagcatgggaagacgctcctgttgca

SEQ ID NO: 64 - DNA, 28 bp, Artificial
  an artificially synthesized sequence
tccaagcgcaatccctgcgcacgaggcg

SEQ ID NO: 65 - DNA, 25 bp, Artificial
  an artificially synthesized sequence
gcctggcctgctgccctcgctggcc

SEQ ID NO: 66 - DNA, 18 bp, Artificial
  an artificially synthesized primer sequence
ctgccaagtatgacatca

SEQ ID NO: 67 - DNA, 21 bp, Artificial
  an artificially synthesized primer sequence
tactccttggaggccatgtag

SEQ ID NO: 68 - DNA, 20 bp, Artificial
  an artificially synthesized primer sequence
gtggatgaggaccacgaact

SEQ ID NO: 69 - DNA, 20 bp, Artificial
  an artificially synthesized primer sequence
cttttcaagcggtggttgat

SEQ ID NO: 70 - DNA, 20 bp, Artificial
  an artificially synthesized primer sequence
acctcctagacccacacacg

SEQ ID NO: 71 - DNA, 20 bp, Artificial
  an artificially synthesized primer sequence
ggatgttggcaaaccagtct

SEQ ID NO: 72 - DNA, 20 bp, Artificial
  an artificially synthesized primer sequence
atgagcccttcaacgaacac

SEQ ID NO: 73 - DNA, 20 bp, Artificial
  an artificially synthesized primer sequence
tggtagaaggggctgatgtc

SEQ ID NO: 74 - DNA, 19 bp, Artificial
  an artificially synthesized primer sequence
ttccaggctttgggcatca

SEQ ID NO: 75 - DNA, 24 bp, Artificial
  an artificially synthesized primer sequence
atgttcagcatgttcagcagtgtg

SEQ ID NO: 76 - DNA, 25 bp, Artificial
  an artificially synthesized primer sequence
catccgtaaagacctctatgccaac

SEQ ID NO: 77 - DNA, 19 bp, Artificial
  an artificially synthesized primer sequence
atggagccaccgatccaca

SEQ ID NO: 78 - DNA, 20 bp, Artificial
  an artificially synthesized primer sequence
tgtgtggacacacctcccta

SEQ ID NO: 79 - DNA, 20 bp, Artificial
  an artificially synthesized primer sequence
cttcaaaggtccccttcctc

SEQ ID NO: 80 - DNA, 20 bp, Artificial
  an artificially synthesized primer sequence
cagcttgagccatttcaaca

SEQ ID NO: 81 - DNA, 20 bp, Artificial
  an artificially synthesized primer sequence
gggtgaggcctttaggaaac

SEQ ID NO: 82 - DNA, 25 bp, Artificial
  an artificially synthesized sequence
gcgccccctctccccatggagaaag

SEQ ID NO: 83 - DNA, 25 bp, Artificial
  an artificially synthesized sequence
gctttgcctcaggatttccgggacc

SEQ ID NO: 84 - DNA, 27 bp, Artificial
  an artificially synthesized sequence
ggttcagccttggtctaccgtgatgtc

SEQ ID NO: 85 - DNA, 25 bp, Artificial
  an artificially synthesized sequence
gcagttgttgctatgcgacctgtat

SEQ ID NO: 86 - DNA, 24 bp, Artificial
  an artificially synthesized sequence
tggggagagtgaggattcggtgaa

SEQ ID NO: 87 - DNA, 27 bp, Artificial
  an artificially synthesized sequence
cggacgtgggactcgtcgaggacaaag

SEQ ID NO: 88 - DNA, 26 bp, Artificial
  an artificially synthesized sequence
cgaaagtacctgcccgcccgtttcgc

SEQ ID NO: 89 - DNA, 21 bp, Artificial
  an artificially synthesized primer sequence
ctgtgagcccaagtgtgtgga

SEQ ID NO: 90 - DNA, 22 bp, Artificial
  an artificially synthesized primer sequence
gtctcgaaacatggcaacagga

SEQ ID NO: 91 - RNA, 27 nt, Artificial
  An artificially synthesized siRNA sequence
gcagcccagcaagaugaauaagaucag

SEQ ID NO: 92 - RNA, 27 nt, Artificial
  An artificially synthesized siRNA sequence
gaucuuauucaucuugcugggcugcau

SEQ ID NO: 93 - DNA, 25 bp, Artificial
  An artificially synthesized primer sequence
catccgtaaagacctctatgccaac

SEQ ID NO: 94 - DNA, 19 bp, Artificial
  An artificially synthesized primer sequence
atggagccaccgatccaca

SEQ ID NO: 95 - DNA, 23 bp, Artificial
  An artificially synthesized primer sequence
caggagggagaacagaaactcca

SEQ ID NO: 96 - DNA, 19 bp, Artificial
  An artificially synthesized primer sequence
cctggttggctgcttgctt

SEQ ID NO: 97 - DNA, 20 bp, Artificial
  An artificially synthesized primer sequence
ctgccctggctatggtcaca

SEQ ID NO: 98 - DNA, 23 bp, Artificial
  An artificially synthesized primer sequence
agacaggtagttgggtcggttca